European Patent Application EP 4 421 086 A1, published August 28, 2024. Title: NUCLEIC ACID VECTOR COMPRISING A CODING SEQUENCE OF THE EPM2A GENE. Applicant: Fundación Instituto de Investigación Sanitaria Fundación Jiménez Díaz. The sequence listing filed with the application follows.

SEQUENCE LISTING (3 sequences)

SEQ ID NO: 1 - DNA, 996 bp, synthetic construct
  source 1..996: mol_type = other DNA
atgcgcttccgctttggggtggtggtgccacccgccgtggccggcgcccggccggagctgctggtggtggggtcgcggcccgagctggggcgttgggagccgcgcggtgccgtccgcctgaggccggccggcaccgcggcgggcgacggggccctggccctgcaggagccgggcctgtggctcggggaggtggagctggcggccgaggaggcggcgcaggacggggcggagccgggccgcgtggacacgttctggtacaagttcctgaagcgggagccgggaggagagctctcctgggaaggcaatggacctcatcatgaccgttgctgtacttacaatgaaaacaacttggtggatggtgtgtattgtctcccaataggacactggattgaggccactgggcacaccaatgaaatgaagcacacaacagacttctattttaatattgcaggccaccaagccatgcattattcaagaattctaccaaatatctggctgggtagctgccctcgtcaggtggaacatgtaaccatcaaactgaagcatgaattggggattacagctgtaatgaatttccagactgaatgggatattgtacagaattcctcaggctgtaaccgctacccagagcccatgactccagacactatgattaaactatatagggaagaaggcttggcctacatctggatgccaacaccagatatgagcaccgaaggccgagtacagatgctgccccaggcggtgtgcctgctgcatgcgctgctggagaagggacacatcgtgtacgtgcactgcaacgctggggtgggccgctccaccgcggctgtctgcggctggctccagtatgtgatgggctggaatctgaggaaggtgcagtatttcctcatggccaagaggccggctgtctacattgacgaagaggccttggcccgggcacaagaagattttttccagaaatttgggaaggttcgttcttctgtgtgtagcctgtag

SEQ ID NO: 2 - protein, 331 aa, synthetic construct
MRFRFGVVVPPAVAGARPELLVVGSRPELGRWEPRGAVRLRPAGTAAGDGALALQEPGLWLGEVELAAEEAAQDGAEPGRVDTFWYKFLKREPGGELSWEGNGPHHDRCCTYNENNLVDGVYCLPIGHWIEATGHTNEMKHTTDFYFNIAGHQAMHYSRILPNIWLGSCPRQVEHVTIKLKHELGITAVMNFQTEWDIVQNSSGCNRYPEPMTPDTMIKLYREEGLAYIWMPTPDMSTEGRVQMLPQAVCLLHALLEKGHIVYVHCNAGVGRSTAAVCGWLQYVMGWNLRKVQYFLMAKRPAVYIDEEALARAQEDFFQKFGKVRSSVCSL

SEQ ID NO: 3 - DNA, 7974 bp, synthetic construct
  source 1..7974: mol_type = other DNA
cagctgcgcgctcgctcgctcactgaggccgcccgggcaaagcccgggcgtcgggcgacctttggtcgcccggcctcagtgagcgagcgagcgcgcagagagggagtggccaactccatcactaggggttccttgtagttaatgattaacccgccatgctacttatctactcgacattgattattgactagttattaatagtaatcaattacggggtcattagttcatagcccatatatggagttccgcgttacataacttacggtaaatggcccgcctggctgaccgcccaacgacccccgcccattgacgtcaataatgacgtatgttcccatagtaacgccaatagggactttccattgacgtcaatgggtggagtatttacggtaaactgcccacttggcagtacatcaagtgtatcatatgccaagtacgccccctattgacgtcaatgacggtaaatggcccgcctggcattatgcccagtacatgaccttatgggactttcctacttggcagtacatctacgtattagtcatcgctattaccatggtcgaggtgagccccacgttctgcttcactctccccatctcccccccctccccacccccaattttgtatttatttattttttaattattttgtgcagcgatgggggcggggggggggggggggcgcgcgccaggcggggcggggcggggcgaggggcggggcggggcgaggcggagaggtgcggcggcagccaatcagagcggcgcgctccgaaagtttccttttatggcgaggcggcggcggcggcggccctataaaaagcgaagcgcgcggcgggcgggagtcgctgcgttgccttcgccccgtgccccgctccgcgccgcctcgcgccgcccgccccggctctgactgaccgcgttactcccacaggtgagcgggcgggacggcccttctcctccgggctgtaattagcgcttggtttaatgacggcttgtttcttttctgtggctgcgtgaaagccttgaggggctccgggagggccctttgtgcggggggagcggctcggggggtgcgtgcgtgtgtgtgtgcgtggggagcgccgcgtgcggctccgcgctgcccggcggctgtgagcgctgcgggcgcggcgcggggctttgtgcgctccgcagtgtgcgcgaggggagcgcggccgggggcggtgccccgcggtgcggggggctgcgaggggaacaaaggctgcgtgcggggtgtgtgcgtgggggggtgagcagggggtgtgggcgcgtcggtcgggctgcaaccccccctgcacccccctccccgagttgctgagcacggcccggcttcgggtgcggggctccgtacggggcgtggcgcggggctcgccgtgccgggcggggggtggcggcaggtgggggtgccgggcggggcggggccgcctcgggccggggagggctcgggggaggggcgcggcggcccccggagcgccggcggctgtcgaggcgcggcgagccgcagccattgccttttatggtaatcgtgcgagagggcgcagggacttcctttgtcccaaatctgtgcggagccgaaatctgggaggcgccgccgcaccccctctagcgggcgcggggcgaagcggtgcggcgccggcaggaaggaaatgggcggggagggccttcgtgcgtcgccgcgccgccgtccccttctccctctccagcctcggggctgtccgcggggggacggctgccttcgggggggacggggcagggcggggttcggcttctggcgtgtgaccggcggctctagagcctctgctaaccatgttcatgccttcttctttttcctacagctcctgggcaacgtgctggttattgtgctgtctcatcattttggcaaagaattgattaattcgagcgaacgcgtcgagtcgctcggtacgatttaaattgaattggcctcgagcgcaagcttgagctagcatgcgcttccgctttggggtggtggtgccacccgccgtggccggcgcccggccggagctgctggtggtggggtcgcggcccgagctggggcgttgggagccgcgcggtgccgtccgcctgaggccggccggcaccgcggcgggcgacggggccctggccctgcaggagccgggcctgtggctcggggaggtggagctggcggccgaggaggcggcgcaggacggggcggagccgggccgcgtggacacgttctggtacaagttcctgaagcgggagccgggaggagagctctcctgggaaggcaatggacctcatcatgaccgttgctgtacttacaatgaaaacaacttggtggatggtgtgtattgtctcccaataggacactggattgaggccactgggcacaccaatgaaatgaagcacacaacagacttctattttaatattgcaggccaccaagccatgcattattcaagaattctaccaaatatctggctgggtagctgccctcgtcaggtggaacatgtaaccatcaaactgaagcatgaattggggattacagctgtaatgaatttccagactgaatgggatattgtacagaattcctcaggctgtaaccgctacccagagcccatgactccagacactatgattaaactatatagggaagaaggcttggcctacatctggatgccaacaccagatatgagcaccgaaggccgagtacagatgctgccccaggcggtgtgcctgctgcatgcgctgctggagaagggacacatcgtgtacgtgcactgcaacgctggggtgggccgctccaccgcggctgtctgcggctggctccagtatgtgatgggctggaatctgaggaaggtgcagtatttcctcatggccaagaggccggctgtctacattgacgaagaggccttggcccgggcacaagaagattttttccagaaatttgggaaggttcgttcttctgtgtgtagcctgtaggcggccgcaagaattcgatatcaagcttatcgataatcaacctctggattacaaaatttgtgaaagattgactggtattcttaactatgttgctccttttacgctatgtggatacgctgctttaatgcctttgtatcatgctattgcttcccgtatggctttcattttctcctccttgtataaatcctggttgctgtctctttatgaggagttgtggcccgttgtcaggcaacgtggcgtggtgtgcactgtgtttgctgacgcaacccccactggttggggcattgccaccacctgtcagctcctttccgggactttcgctttccccctccctattgccacggcggaactcatcgccgcctgccttgcccgctgctggacaggggctcggctgttgggcactgacaattccgtggtgttgtcggggaaatcatcgtcctttccttggctgctcgcctgtgttgccacctggattctgcgcgggacgtccttctgctacgtcccttcggccctcaatccagcggaccttccttcccgcggcctgctgccggctctgcggcctcttccgcgtcttcgccttcgccctcagacgagtcggatctccctttgggccgcctccccgcctgatcgataccgtcgacctcgagggggggcccggtacccgggaatcaattcactcctcaggtgcaggctgcctatcagaaggtggtggctggtgtggccaatgccctggctcacaaataccactgagatctttttccctctgccaaaaattatggggacatcatgaagccccttgagcatctgacttctggctaataaaggaaatttattttcattgcaatagtgtgttggaattttttgtgtctctcactcggaaggacatatgggagggcaaatcatttaaaacatcagaatgagtatttggtttagagtttggcaacatatgcccatatgctggctgccatgaacaaaggttggctataaagaggtcatcagtatatgaaacagccccctgctgtccattccttattccatagaaaagccttgacttgaggttagattttttttatattttgttttgtgttatttttttctttaacatccctaaaattttccttacatgttttactagccagatttttcctcctctcctgactactcccagtcatagctgtccctcttctcttatggagatccctcgacctgcagcccaagctgtagataagtagcatggcgggttaatcattaactacaaggaacccctagtgatggagttggccactccctctctgcgcgctcgctcgctcactgaggccgggcgaccaaaggtcgcccgacgcccgggctttgcccgggcggcctcagtgagcgagcgagcgcgcagctggcgtaatagcgaagaggcccgcaccgatcgcccttcccaacagttgcgcagcctgaatggcgaatggcgattccgttgcaatggctggcggtaatattgttctggatattaccagcaaggccgatagtttgagttcttctactcaggcaagtgatgttattactaatcaaagaagtattgcgacaacggttaatttgcgtgatggacagactcttttactcggtggcctcactgattataaaaacacttctcaggattctggcgtaccgttcctgtctaaaatccctttaatcggcctcctgtttagctcccgctctgattctaacgaggaaagcacgttatacgtgctcgtcaaagcaaccatagtacgcgccctgtagcggcgcattaagcgcggcgggtgtggtggttacgcgcagcgtgaccgctacacttgccagcgccctagcgcccgctcctttcgctttcttcccttcctttctcgccacgttcgccggctttccccgtcaagctctaaatcgggggctccctttagggttccgatttagtgctttacggcacctcgaccccaaaaaacttgattagggtgatggttcacgtagtgggccatcgccctgatagacggtttttcgccctttgacgttggagtccacgttctttaatagtggactcttgttccaaactggaacaacactcaaccctatctcggtctattcttttgatttataagggattttgccgatttcggcctattggttaaaaaatgagctgatttaacaaaaatttaacgcgaattttaacaaaatattaacgcttacaatttaaatatttgcttatacaatcttcctgtttttggggcttttctgattatcaaccggggtacatatgattgacatgctagttttacgattaccgttcatcgattctcttgtttgctccagactctcaggcaatgacctgatagcctttgtagagacctctcaaaaatagctaccctctccggcatgaatttatcagctagaacggttgaatatcatattgatggtgatttgactgtctccggcctttctcacccgtttgaatctttacctacacattactcaggcattgcatttaaaatatatgagggttctaaaaatttttatccttgcgttgaaataaaggcttctcccgcaaaagtattacagggtcataatgtttttggtacaaccgatttagctttatgctctgaggctttattgcttaattttgctaattctttgccttgcctgtatgatttattggatgttggaatcgcctgatgcggtattttctccttacgcatctgtgcggtatttcacaccgcatatggtgcactctcagtacaatctgctctgatgccgcatagttaagccagccccgacacccgccaacacccgctgacgcgccctgacgggcttgtctgctcccggcatccgcttacagacaagctgtgaccgtctccgggagctgcatgtgtcagaggttttcaccgtcatcaccgaaacgcgcgagacgaaagggcctcgtgatacgcctatttttataggttaatgtcatgataataatggtttcttagacgtcaggtggcacttttcggggaaatgtgcgcggaacccctatttgtttatttttctaaatacattcaaatatgtatccgctcatgagacaataaccctgataaatgcttcaataatattgaaaaaggaagagtatgagtattcaacatttccgtgtcgcccttattcccttttttgcggcattttgccttcctgtttttgctcacccagaaacgctggtgaaagtaaaagatgctgaagatcagttgggtgcacgagtgggttacatcgaactggatctcaacagcggtaagatccttgagagttttcgccccgaagaacgttttccaatgatgagcacttttaaagttctgctatgtggcgcggtattatcccgtattgacgccgggcaagagcaactcggtcgccgcatacactattctcagaatgacttggttgagtactcaccagtcacagaaaagcatcttacggatggcatgacagtaagagaattatgcagtgctgccataaccatgagtgataacactgcggccaacttacttctgacaacgatcggaggaccgaaggagctaaccgcttttttgcacaacatgggggatcatgtaactcgccttgatcgttgggaaccggagctgaatgaagccataccaaacgacgagcgtgacaccacgatgcctgtagcaatggcaacaacgttgcgcaaactattaactggcgaactacttactctagcttcccggcaacaattaatagactggatggaggcggataaagttgcaggaccacttctgcgctcggcccttccggctggctggtttattgctgataaatctggagccggtgagcgtgggtctcgcggtatcattgcagcactggggccagatggtaagccctcccgtatcgtagttatctacacgacggggagtcaggcaactatggatgaacgaaatagacagatcgctgagataggtgcctcactgattaagcattggtaactgtcagaccaagtttactcatatatactttagattgatttaaaacttcatttttaatttaaaaggatctaggtgaagatcctttttgataatctcatgaccaaaatcccttaacgtgagttttcgttccactgagcgtcagaccccgtagaaaagatcaaaggatcttcttgagatcctttttttctgcgcgtaatctgctgcttgcaaacaaaaaaaccaccgctaccagcggtggtttgtttgccggatcaagagctaccaactctttttccgaaggtaactggcttcagcagagcgcagataccaaatactgttcttctagtgtagccgtagttaggccaccacttcaagaactctgtagcaccgcctacatacctcgctctgctaatcctgttaccagtggctgctgccagtggcgataagtcgtgtcttaccgggttggactcaagacgatagttaccggataaggcgcagcggtcgggctgaacggggggttcgtgcacacagcccagcttggagcgaacgacctacaccgaactgagatacctacagcgtgagctatgagaaagcgccacgcttcccgaagggagaaaggcggacaggtatccggtaagcggcagggtcggaacaggagagcgcacgagggagcttccagggggaaacgcctggtatctttatagtcctgtcgggtttcgccacctctgacttgagcgtcgatttttgtgatgctcgtcaggggggcggagcctatggaaaaacgccagcaacgcggcctttttacggttcctggccttttgctggccttttgctcacatgttctttcctgcgttatcccctgattctgtggataaccgtattaccgcctttgagtgagctgataccgctcgccgcagccgaacgaccgagcgcagcgagtcagtgagcgaggaagcggaagagcgcccaatacgcaaaccgcctctccccgcgcgttggccgattcattaatgcagctgcgcgctcgctcgctcactgaggcc